European Patent Specification EP 3 360 899 B1, published January 25, 2023. Title: ANTIBODIES TO CARCINOEMBRYONIC ANTIGEN-RELATED CELL ADHESION MOLECULE (CEACAM). Applicant: Tel Hashomer Medical Research Infrastructure and Services Ltd CCAM BIOTHERAPEUTICS LTD. The sequence listing filed with the application follows.

SEQUENCE LISTING (35 sequences)

SEQ ID NO: 1 - protein, 5 aa, Mus musculus
  MISC_FEATURE (1)..(1): X is Absent or Thr
  MISC_FEATURE (5)..(5): X is Absent or Ile
XNNLX

SEQ ID NO: 2 - protein, 8 aa, Mus musculus
INPGSGDT

SEQ ID NO: 3 - protein, 11 aa, Mus musculus
GDYYGGFAVDY

SEQ ID NO: 4 - protein, 6 aa, Mus musculus
QDIGNY

SEQ ID NO: 5 - protein, 4 aa, Mus musculus
YTSR

SEQ ID NO: 6 - protein, 7 aa, Mus musculus
QQGKSLP

SEQ ID NO: 7 - protein, 5 aa, Mus musculus
NNLIE

SEQ ID NO: 8 - protein, 17 aa, Mus musculus
VINPGSGDTNYNEKFKG

SEQ ID NO: 9 - protein, 11 aa, Mus musculus
GDYYGGFAVDY

SEQ ID NO: 10 - protein, 11 aa, Mus musculus
RTSQDIGNYLN

SEQ ID NO: 11 - protein, 7 aa, Mus musculus
YTSRLHS

SEQ ID NO: 12 - protein, 7 aa, Mus musculus
QQGKSLP

SEQ ID NO: 13 - protein, 8 aa, Mus musculus
GYAFTNNL

SEQ ID NO: 14 - protein, 8 aa, Mus musculus
INPGSGDT

SEQ ID NO: 15 - protein, 13 aa, Mus musculus
ARGDYYGGFAVDY

SEQ ID NO: 16 - protein, 6 aa, Mus musculus
QDIGNY

SEQ ID NO: 17 - protein, 4 aa, Mus musculus
YTSR

SEQ ID NO: 18 - protein, 9 aa, Mus musculus
QQGKSLPRT

SEQ ID NO: 19 - protein, 10 aa, Mus musculus
GYAFTNNLIE

SEQ ID NO: 20 - protein, 17 aa, Mus musculus
VINPGSGDTNYNEKFKG

SEQ ID NO: 21 - protein, 13 aa, Mus musculus
ARGDYYGGFAVDY

SEQ ID NO: 22 - protein, 11 aa, Mus musculus
RTSQDIGNYLN

SEQ ID NO: 23 - protein, 7 aa, Mus musculus
YTSRLHS

SEQ ID NO: 24 - protein, 9 aa, Mus musculus
QQGKSLPRT

SEQ ID NO: 25 - DNA, 467 bp, artificial sequence
  Recombinant DNA
atgggatggaccttggtctttctctttctcctgtcagtaactgcaggtgttcactcccaggtccagctgcagcagtctggagctgagctggtaaggcctgggacttcagtgaaggtgtcctgcaaggcttctggatacgccttcactaataacttgatagagtgggtaaaacagaggcctggacagggccttgagtggattggagtgattaatcctggaagtggtgatactaactacaatgagaagttcaagggcaaggcaacactgactgcagacaaatcctccaacactgcctacatgcagctcagcagcctgacatctgatgactctgcggtctatttctgtgcaagaggggattactacggtggctttgctgtggactactggggtcaaggaacctcagtcaccgtctcctcagccaaaacgacacccccatccgtttatcccttggcccctggaagcttggg

SEQ ID NO: 26 - protein, 120 aa, artificial sequence
  Recombinant polypeptide
QVQLQQSGAELVRPGTSVKVSCKASGYAFTNNLIEWVKQRPGQGLEWIGVINPGSGDTNYNEKFKGKATLTADKSSNTAYMQLSSLTSDDSAVYFCARGDYYGGFAVDYWGQGTSVTVSS

SEQ ID NO: 27 - DNA, 488 bp, artificial sequence
  Recombinant DNA
atggtgtcctcagctcagttccttggtctcctgttgctctgttttcaaggaaccagatgtgatatccagatgacacagactacatcctccctgtctgcctctctgggagacagagtcaccatcagttgcaggacaagtcaggacattggcaattatttaaactggtatcagcagaaaccagatggaactgttaaactcctgatctactacacatcaagattacactcaggagtcccatcaaggttcagtggcagtgggtctggaacagattattctctcaccattagcaacctggagcaagaagatattgccacttacttttgccaacagggtaaaagccttcctcggacgttcggtggaggcaccaagttggaaatcaaacgggctgatgctgcaccaactgtatccatcttcccaccatccagtgagcagttaacatctggaggtgcctcagtcgtgtgcttcttgaacaacttctaccccagaga

SEQ ID NO: 28 - protein, 107 aa, artificial sequence
  Recombinant polypeptide
DIQMTQTTSSLSASLGDRVTISCRTSQDIGNYLNWYQQKPDGTVKLLIYYTSRLHSGVPSRFSGSGSGTDYSLTISNLEQEDIATYFCQQGKSLPRTFGGGTKLEIK

SEQ ID NO: 29 - protein, 10 aa, artificial sequence
  Recombinant peptide
DIQMTQTTSS

SEQ ID NO: 30 - protein, 450 aa, artificial sequence
  Recombinant polypeptide
QVQLQQSGAELVRPGTSVKVSCKASGYAFTNNLIEWVKQRPGQGLEWIGVINPGSGDTNYNEKFKGKATLTADKSSNTAYMQLSSLTSDDSAVYFCARGDYYGGFAVDYWGQGTSVTVSSASTKGPSVFPLAPSSKSTSGGTAALGCLVKDYFPEPVTVSWNSGALTSGVHTFPAVLQSSGLYSLSSVVTVPSSSLGTQTYICNVNHKPSNTKVDKKVEPKSCDKTHTCPPCPAPELLGGPSVFLFPPKPKDTLMISRTPEVTCVVVDVSHEDPEVKFNWYVDGVEVHNAKTKPREEQYNSTYRVVSVLTVLHQDWLNGKEYKCKVSNKALPAPIEKTISKAKGQPREPQVYTLPPSRDELTKNQVSLTCLVKGFYPSDIAVEWESNGQPENNYKTTPPVLDSDGSFFLYSKLTVDKSRWQQGNVFSCSVMHEALHNHYTQKSLSLSPGK

SEQ ID NO: 31 - protein, 214 aa, artificial sequence
  Recombinant polypeptide
DIQMTQTTSSLSASLGDRVTISCRTSQDIGNYLNWYQQKPDGTVKLLIYYTSRLHSGVPSRFSGSGSGTDYSLTISNLEQEDIATYFCQQGKSLPRTFGGGTKLEIKRTVAAPSVFIFPPSDEQLKSGTASVVCLLNNFYPREAKVQWKVDNALQSGNSQESVTEQDSKDSTYSLSSTLTLSKADYEKHKVYACEVTHQGLSSPVTKSFNRGEC

SEQ ID NO: 32 - protein, 13 aa, Homo sapiens
VLLLVHNLPQQLF

SEQ ID NO: 33 - protein, 12 aa, Homo sapiens
YPNASLLIQNVT

SEQ ID NO: 34 - protein, 7 aa, Homo sapiens
PNASLLI

SEQ ID NO: 35 - protein, 108 aa, Homo sapiens
QLTTESMPFNVAEGKEVLLLVHNLPQQLFGYSWYKGERVDGNRQIVGYAIGTQQATPGPANSGRETIYPNASLLIQNVTQNDTGFYTLQVIKSDLVNEEATGQFHVYP